European Patent Application EP 4 628 506 A1, published October 8, 2025. Title: PREPARATION METHOD FOR AND USE OF CD70-SPECIFIC INTEGRATED DIAGNOSIS AND TREATMENT MOLECULAR IMAGING PROBE. Applicant: RENJI HOSPITAL, SHANGHAI JIAO TONG UNIVERSITY SCHOOL OF MEDICINE. The sequence listing filed with the application follows.

SEQUENCE LISTING (10 sequences)

SEQ ID NO: 1 - protein, 152 aa, synthetic construct
QVQLQESGGGSVQAGGSLRLSCAASGIIVNDGCMAWFRQVPGKEREGVAGIVIGEYGGGTTYYADSVKGRFTISRDRAKNTLYLQMNSLKPEDTAMYYCAADQWASGGCTSIATFSDEFDYWGQGTQVTVSSGGGGSGGGGSLLQSHHHHHH

SEQ ID NO: 2 - DNA, 456 bp, synthetic construct
  source 1..456: mol_type = other DNA
caggttcagctccaggaaagcggaggaggaagcgttcaggcaggaggatctctcaggctctcctgtgctgcatcaggcatcatcgtcaacgacggctgcatggcttggttcaggcaggttcctggcaaagagagggaaggggtggctggaattgtcattggggagtacggcggcggaaccacatattacgccgactctgtgaagggaaggttcaccatctcccgggacagggctaagaacaccctgtatttgcagatgaactctctgaagcccgaggacaccgccatgtattactgcgcagccgaccagtgggcctctggaggatgtacatccatcgccaccttttccgatgagttcgactattggggacagggcacacaggtcaccgtgtctagtggtggaggaggttctggaggtggtggatcattgctgcagtcccaccatcaccatcatcac

SEQ ID NO: 3 - protein, 151 aa, synthetic construct
QVQLQESGGGSVQAGGSLRLSCVASDLIVNDGCMAWFRQVPGKEHEGVARIAIPTTPGSTLYADSVKGRFTISRDGAKNTLYLQMNSLKPEDTAVYYCAADQWASRGCTAIATIPAEFDYWGQGTQVTVSSGGGGSGGGGSLLQSHHHHHH

SEQ ID NO: 4 - DNA, 453 bp, synthetic construct
  source 1..453: mol_type = other DNA
caggttcagctccaggaaagcggaggaggaagcgttcaggcaggaggatctctcaggctctcctgtgtggcatccgacttgatcgtcaacgacggctgcatggcctggttcagacaggttcctggcaaagagcacgagggggttgctagaattgcaatccctacaacccccggatctaccctgtatgccgactctgtgaagggaaggtttacaatctccagagacggcgccaagaataccctgtacctgcagatgaacagtctgaaacccgaagatactgctgtgtactactgcgccgccgaccagtgggcttctaggggatgtactgccatcgccacaattcctgccgaatttgactattggggccagggaacccaggttaccgttagttccggtggaggaggttctggaggtggtggatcattgctgcagtcccaccatcaccatcatcac

SEQ ID NO: 5 - protein, 208 aa, synthetic construct
HHHHHHQVQLQESGGGSVQAGGSLRLSCAASGIIVNDGCMAWFRQVPGKEREGVAGIVIGEYGGGTTYYADSVKGRFTISRDRAKNTLYLQMNSLKPEDTAMYYCAADQWASGGCTSIATFSDEFDYWGQGTQVTVSSGGGGSGGGGSGGGGSLAEAKVLANRELDKYGVSDFYKRLINKAKTVEGVEALKLHILAALPGGGGSLLQS

SEQ ID NO: 6 - DNA, 624 bp, synthetic construct
  source 1..624: mol_type = other DNA
caccatcaccaccaccatcaggtgcagctgcaggaaagcggaggaggatctgtgcaggctggaggatcactgagactgagctgtgccgcttccggaatcatcgtgaacgacggatgcatggcctggttcagacaggtgcctggaaaagagagagagggggtggctggaattgtgattggagagtacggcgggggaaccacttattatgccgacagcgtgaagggaagatttactatcagcagagacagagccaagaacacactgtacctgcagatgaatagtctgaagcccgaggatacagccatgtactactgcgccgccgaccagtgggcttccggaggatgcaccagcattgctacatttagcgatgagttcgactactggggccagggaacacaggtgacagtgtctagcggtggtggcggatcaggtgggggaggctctggtggaggcggtagtctggctgaagctaaagtgctggctaacagagagctggacaaatacggcgtgagcgacttctataaaagactgatcaacaaggccaagaccgtggaaggcgtggaggctctgaagctgcatatcctggctgccctgcctggaggaggaggaagcctgctgcagagc

SEQ ID NO: 7 - protein, 207 aa, synthetic construct
HHHHHHQVQLQESGGGSVQAGGSLRLSCVASDLIVNDGCMAWFRQVPGKEHEGVARIAIPTTPGSTLYADSVKGRFTISRDGAKNTLYLQMNSLKPEDTAVYYCAADQWASRGCTAIATIPAEFDYWGQGTQVTVSSGGGGSGGGGSGGGGSLAEAKVLANRELDKYGVSDFYKRLINKAKTVEGVEALKLHILAALPGGGGSLLQS

SEQ ID NO: 8 - DNA, 621 bp, synthetic construct
  source 1..621: mol_type = other DNA
caccatcaccaccaccatcaggtgcagctgcaggagagcggaggaggaagcgtgcaggctggaggaagcctgaggctgagctgcgtggcttccgacctgattgtgaacgacggctgcatggcctggttcagacaggtgcctggaaaagaacacgagggggtggctagaattgccatccctacaacacccggatctacactgtatgccgactccgtgaagggaagatttacaatcagcagagatggcgccaaaaacaccctgtacctgcagatgaacagcctgaagcccgaagatactgctgtgtactactgcgccgccgaccagtgggcttccaggggatgcaccgctattgctaccattcctgccgaatttgactattggggccagggcacccaggtgaccgtgagcagcggtggtggcggatcaggtgggggaggctctggtggaggcggtagtctggctgaagctaaagtgctggctaacagagagctggacaaatacggcgtgagcgacttctataaaagactgatcaacaaggccaagaccgtggaaggcgtggaggctctgaagctgcatatcctggctgccctgcctggaggaggaggaagcctgctgcagagc

SEQ ID NO: 9 - protein, 15 aa, synthetic construct
GGGGSGGGGSGGGGS

SEQ ID NO: 10 - DNA, 45 bp, synthetic construct
  source 1..45: mol_type = other DNA
ggtggtggcggatcaggtgggggaggctctggtggaggcggtagt